European Patent Application EP 4 563 160 A1, published June 4, 2025. Title: Agent for treating lung adenocarcinoma. Applicant: Keio University. The sequence listing filed with the application follows.

SEQUENCE LISTING (2 sequences)

SEQ ID NO: 1 - DNA, 29 bp, Homo sapiens
  source 1..29: mol_type = genomic DNA
ctggaggaaagctacaagaaagtgggcat

SEQ ID NO: 2 - DNA, 25 bp, Homo sapiens
  source 1..25: mol_type = genomic DNA
ctggaggaaagctacaagtgggcat